European Patent Specification EP 3 424 955 B1, published April 9, 2025. Title: ANTI-TROP2 ANTIBODY-DRUG CONJUGATE. Applicant: Daiichi Sankyo Company, Limited. Application EP14874745.4. The sequence listing filed with the application follows.

SEQUENCE LISTING (54 sequences)

SEQ ID NO: 1 - DNA, 363 bp, Mus musculus
cagatccagttggtgcagtctggacctgagctgaagaagcctggagagacagtcaggatctcctgcaaggcttctgggtataccttcacaactgctggaatgcagtgggtgcaaaagatgccaggaaagggtttgaagtggattggctggataaacacccactctggagtgccaaaatatgcagaagacttcaagggacggtttgccttctctttggaaacctctgccagcactgcatatttacagataagcaacctcaaaaatgaggacacgactacgtatttctgtgcgagatcggggttcggtagtagctactggtacttcgatgtctggggcgcagggaccgcggtcaccgtctcctca

SEQ ID NO: 2 - protein, 121 aa, Mus musculus
QIQLVQSGPELKKPGETVRISCKASGYTFTTAGMQWVQKMPGKGLKWIGWINTHSGVPKYAEDFKGRFAFSLETSASTAYLQISNLKNEDTTTYFCARSGFGSSYWYFDVWGAGTAVTVSS

SEQ ID NO: 3 - DNA, 327 bp, Mus musculus
gacattgtgatgacccagtctcacaaattcatgtccacatcagtaggagacagggtcagcatcacctgcaaggccagtcaggatgtgagtactgctgtagcctggtatcaacagaaaccaggacaatctcctaaactgctgatttactcggcatcctaccgctacactggagtccctgatcgcttcactggcagtggatctgggacggctttcactttcaccatcagcagtgtgcaggctgaagacctggcagtttattactgtcagcaacattatattactccgctcacgttcggtgctgggaccaagctggagctgaaacgggct

SEQ ID NO: 4 - protein, 109 aa, Mus musculus
DIVMTQSHKFMSTSVGDRVSITCKASQDVSTAVAWYQQKPGQSPKLLIYSASYRYTGVPDRFTGSGSGTAFTFTISSVQAEDLAVYYCQQHYITPLTFGAGTKLELKRA

SEQ ID NO: 5 - DNA, 449 bp, Homo sapiens
gcctccggactctagagccaccatggtgctgcagacccaggtgttcatctccctgctgctgtggatctccggcgcgtacggcgatatcgtgatgattaaacgtacggtggccgccccctccgtgttcatcttccccccctccgacgagcagctgaagtccggcaccgcctccgtggtgtgcctgctgaataacttctaccccagagaggccaaggtgcagtggaaggtggacaacgccctgcagtccgggaactcccaggagagcgtgaccgagcaggacagcaaggacagcacctacagcctgagcagcaccctgaccctgagcaaagccgactacgagaagcacaaggtgtacgcctgcgaggtgacccaccagggcctgagctcccccgtcaccaagagcttcaacaggggggagtgttaggggcccgtttaaacgggggaggcta

SEQ ID NO: 6 - DNA, 1132 bp, Homo sapiens
gcctccggactctagagccaccatgaaacacctgtggttcttcctcctgctggtggcagctcccagatgggtgctgagccaggtgcaattgtgcaggcggttagctcagcctccaccaagggcccaagcgtcttccccctggcaccctcctccaagagcacctctggcggcacagccgccctgggctgcctggtcaaggactacttccccgaacccgtgaccgtgagctggaactcaggcgccctgaccagcggcgtgcacaccttccccgctgtcctgcagtcctcaggactctactccctcagcagcgtggtgaccgtgccctccagcagcttgggcacccagacctacatctgcaacgtgaatcacaagcccagcaacaccaaggtggacaagagagttgagcccaaatcttgtgacaaaactcacacatgcccaccctgcccagcacctgaactcctggggggaccctcagtcttcctcttccccccaaaacccaaggacaccctcatgatctcccggacccctgaggtcacatgcgtggtggtggacgtgagccacgaagaccctgaggtcaagttcaactggtacgtggacggcgtggaggtgcataatgccaagacaaagccccgggaggagcagtacaacagcacgtaccgggtggtcagcgtcctcaccgtcctgcaccaggactggctgaatggcaaggagtacaagtgcaaggtctccaacaaagccctcccagcccccatcgagaaaaccatctccaaagccaaaggccagccccgggaaccacaggtgtacaccctgcccccatcccgggaggagatgaccaagaaccaggtcagcctgacctgcctggtcaaaggcttctatcccagcgacatcgccgtggagtgggagagcaatggccagcccgagaacaactacaagaccacccctcccgtgctggactccgacggctccttcttcctctacagcaagctcaccgtggacaagagcaggtggcagcagggcaacgtcttctcatgctccgtgatgcatgaggctctgcacaaccactacacccagaagagcctctccctgtctcccggcaaatgagatatcgggcccgtttaaacgggggaggcta

SEQ ID NO: 7 - DNA, 1410 bp, Artificial Sequence
  nucleotide sequence of heavy chain of chimeric murine-human TINA1 antibody
atgaaacacctgtggttcttcctcctgctggtggcagctcccagatgggtgctgagccagatccagttggtgcagtctggacctgagctgaagaagcctggagagacagtcaggatctcctgcaaggcttctgggtataccttcacaactgctggaatgcagtgggtgcaaaagatgccaggaaagggtttgaagtggattggctggataaacacccactctggagtgccaaaatatgcagaagacttcaagggacggtttgccttctctttggaaacctctgccagcactgcatatttacagataagcaacctcaaaaatgaggacacgactacgtatttctgtgcgagatcggggttcggtagtagctactggtacttcgatgtctggggcgcagggaccgcggtcaccgtcagctcagcctccaccaagggcccaagcgtcttccccctggcaccctcctccaagagcacctctggcggcacagccgccctgggctgcctggtcaaggactacttccccgaacccgtgaccgtgagctggaactcaggcgccctgaccagcggcgtgcacaccttccccgctgtcctgcagtcctcaggactctactccctcagcagcgtggtgaccgtgccctccagcagcttgggcacccagacctacatctgcaacgtgaatcacaagcccagcaacaccaaggtggacaagagagttgagcccaaatcttgtgacaaaactcacacatgcccaccctgcccagcacctgaactcctggggggaccctcagtcttcctcttccccccaaaacccaaggacaccctcatgatctcccggacccctgaggtcacatgcgtggtggtggacgtgagccacgaagaccctgaggtcaagttcaactggtacgtggacggcgtggaggtgcataatgccaagacaaagccccgggaggagcagtacaacagcacgtaccgggtggtcagcgtcctcaccgtcctgcaccaggactggctgaatggcaaggagtacaagtgcaaggtctccaacaaagccctcccagcccccatcgagaaaaccatctccaaagccaaaggccagccccgggaaccacaggtgtacaccctgcccccatcccgggaggagatgaccaagaaccaggtcagcctgacctgcctggtcaaaggcttctatcccagcgacatcgccgtggagtgggagagcaatggccagcccgagaacaactacaagaccacccctcccgtgctggactccgacggctccttcttcctctacagcaagctcaccgtggacaagagcaggtggcagcagggcaacgtcttctcatgctccgtgatgcatgaggctctgcacaaccactacacccagaagagcctctccctgtctcccggcaaa

SEQ ID NO: 8 - protein, 470 aa, Artificial Sequence
  amino acid sequence of heavy chain of chimeric murine-human TINA1 antibody
MKHLWFFLLLVAAPRWVLSQIQLVQSGPELKKPGETVRISCKASGYTFTTAGMQWVQKMPGKGLKWIGWINTHSGVPKYAEDFKGRFAFSLETSASTAYLQISNLKNEDTTTYFCARSGFGSSYWYFDVWGAGTAVTVSSASTKGPSVFPLAPSSKSTSGGTAALGCLVKDYFPEPVTVSWNSGALTSGVHTFPAVLQSSGLYSLSSVVTVPSSSLGTQTYICNVNHKPSNTKVDKRVEPKSCDKTHTCPPCPAPELLGGPSVFLFPPKPKDTLMISRTPEVTCVVVDVSHEDPEVKFNWYVDGVEVHNAKTKPREEQYNSTYRVVSVLTVLHQDWLNGKEYKCKVSNKALPAPIEKTISKAKGQPREPQVYTLPPSREEMTKNQVSLTCLVKGFYPSDIAVEWESNGQPENNYKTTPPVLDSDGSFFLYSKLTVDKSRWQQGNVFSCSVMHEALHNHYTQKSLSLSPGK

SEQ ID NO: 9 - DNA, 702 bp, Artificial Sequence
  nucleotide sequence of light chain of chimeric murine-human TINA1 antibody
atggtgctgcagacccaggtgttcatctccctgctgctgtggatctccggcgcgtacggcgacattgtgatgacccagtctcacaaattcatgtccacatcagtaggagacagggtcagcatcacctgcaaggccagtcaggatgtgagtactgctgtagcctggtatcaacagaaaccaggacaatctcctaaactgctgatttactcggcatcctaccgctacactggagtccctgatcgcttcactggcagtggatctgggacggctttcactttcaccatcagcagtgtgcaggctgaagacctggcagtttattactgtcagcaacattatattactccgctcacgttcggtgctgggaccaagctggagctgaaacgggctgtggccgccccctccgtgttcatcttccccccctccgacgagcagctgaagtccggcaccgcctccgtggtgtgcctgctgaataacttctaccccagagaggccaaggtgcagtggaaggtggacaacgccctgcagtccgggaactcccaggagagcgtgaccgagcaggacagcaaggacagcacctacagcctgagcagcaccctgaccctgagcaaagccgactacgagaagcacaaggtgtacgcctgcgaggtgacccaccagggcctgagctcccccgtcaccaagagcttcaacaggggggagtgt

SEQ ID NO: 10 - protein, 234 aa, Artificial Sequence
  amino acid sequence of light chain of chimeric murine-human TINA1 antibody
MVLQTQVFISLLLWISGAYGDIVMTQSHKFMSTSVGDRVSITCKASQDVSTAVAWYQQKPGQSPKLLIYSASYRYTGVPDRFTGSGSGTAFTFTISSVQAEDLAVYYCQQHYITPLTFGAGTKLELKRAVAAPSVFIFPPSDEQLKSGTASVVCLLNNFYPREAKVQWKVDNALQSGNSQESVTEQDSKDSTYSLSSTLTLSKADYEKHKVYACEVTHQGLSSPVTKSFNRGEC

SEQ ID NO: 11 - DNA, 1410 bp, Artificial Sequence
  nucleotide sequence of heavy chain of humanized TINA1 antibody, type H1
atgaaacacctgtggttcttcctcctgctggtggcagctcccagatgggtgctgagccaggtgcagctggtgcagtctggcgccgaagtgaagaaaccaggcgccagcgtgaaggtgtcctgcaaggccagcggctacacctttaccaccgccggcatgcagtgggtgcgccaggctcctggacagggcctggaatggatgggctggatcaacacccacagcggcgtgcccaaatacgccgaggacttcaagggcagagtgaccatcagcgccgacaccagcacctccacagcctacctgcagctgagcagcctgaagtccgaggacaccgccgtgtactactgcgccagaagcggcttcggcagcagctactggtacttcgacgtgtggggccagggcaccctcgtgaccgtcagctcagcctccaccaagggcccaagcgtcttccccctggcaccctcctccaagagcacctctggcggcacagccgccctgggctgcctggtcaaggactacttccccgaacccgtgaccgtgagctggaactcaggcgccctgaccagcggcgtgcacaccttccccgctgtcctgcagtcctcaggactctactccctcagcagcgtggtgaccgtgccctccagcagcttgggcacccagacctacatctgcaacgtgaatcacaagcccagcaacaccaaggtggacaagagagttgagcccaaatcttgtgacaaaactcacacatgcccaccctgcccagcacctgaactcctggggggaccctcagtcttcctcttccccccaaaacccaaggacaccctcatgatctcccggacccctgaggtcacatgcgtggtggtggacgtgagccacgaagaccctgaggtcaagttcaactggtacgtggacggcgtggaggtgcataatgccaagacaaagccccgggaggagcagtacaacagcacgtaccgggtggtcagcgtcctcaccgtcctgcaccaggactggctgaatggcaaggagtacaagtgcaaggtctccaacaaagccctcccagcccccatcgagaaaaccatctccaaagccaaaggccagccccgggaaccacaggtgtacaccctgcccccatcccgggaggagatgaccaagaaccaggtcagcctgacctgcctggtcaaaggcttctatcccagcgacatcgccgtggagtgggagagcaatggccagcccgagaacaactacaagaccacccctcccgtgctggactccgacggctccttcttcctctacagcaagctcaccgtggacaagagcaggtggcagcagggcaacgtcttctcatgctccgtgatgcatgaggctctgcacaaccactacacccagaagagcctctccctgtctcccggcaaa

SEQ ID NO: 12 - protein, 470 aa, Artificial Sequence
  amino acid sequence of heavy chain of humanized TINA1 antibody, type H1
MKHLWFFLLLVAAPRWVLSQVQLVQSGAEVKKPGASVKVSCKASGYTFTTAGMQWVRQAPGQGLEWMGWINTHSGVPKYAEDFKGRVTISADTSTSTAYLQLSSLKSEDTAVYYCARSGFGSSYWYFDVWGQGTLVTVSSASTKGPSVFPLAPSSKSTSGGTAALGCLVKDYFPEPVTVSWNSGALTSGVHTFPAVLQSSGLYSLSSVVTVPSSSLGTQTYICNVNHKPSNTKVDKRVEPKSCDKTHTCPPCPAPELLGGPSVFLFPPKPKDTLMISRTPEVTCVVVDVSHEDPEVKFNWYVDGVEVHNAKTKPREEQYNSTYRVVSVLTVLHQDWLNGKEYKCKVSNKALPAPIEKTISKAKGQPREPQVYTLPPSREEMTKNQVSLTCLVKGFYPSDIAVEWESNGQPENNYKTTPPVLDSDGSFFLYSKLTVDKSRWQQGNVFSCSVMHEALHNHYTQKSLSLSPGK

SEQ ID NO: 13 - DNA, 1410 bp, Artificial Sequence
  nucleotide sequence of heavy chain of humanized TINA1 antibody, type H2
atgaaacacctgtggttcttcctcctgctggtggcagctcccagatgggtgctgagccaggtgcagctggtgcagtctggcgccgaagtgaagaaaccaggcgccagcgtgaaggtgtcctgcaaggccagcggctacacctttaccaccgccggcatgcagtgggtgcgccaggctcctggacagggcctggaatggatgggctggatcaacacccacagcggcgtgcccaaatacgccgaggacttcaagggcagagtgaccatcagcctggacaccagcacctccaccgcctacctgcagctgagcagcctgaagtccgaggacaccgccgtgtactactgcgccagaagcggcttcggcagcagctactggtacttcgacgtgtggggccagggcaccctcgtgaccgtcagctcagcctccaccaagggcccaagcgtcttccccctggcaccctcctccaagagcacctctggcggcacagccgccctgggctgcctggtcaaggactacttccccgaacccgtgaccgtgagctggaactcaggcgccctgaccagcggcgtgcacaccttccccgctgtcctgcagtcctcaggactctactccctcagcagcgtggtgaccgtgccctccagcagcttgggcacccagacctacatctgcaacgtgaatcacaagcccagcaacaccaaggtggacaagagagttgagcccaaatcttgtgacaaaactcacacatgcccaccctgcccagcacctgaactcctggggggaccctcagtcttcctcttccccccaaaacccaaggacaccctcatgatctcccggacccctgaggtcacatgcgtggtggtggacgtgagccacgaagaccctgaggtcaagttcaactggtacgtggacggcgtggaggtgcataatgccaagacaaagccccgggaggagcagtacaacagcacgtaccgggtggtcagcgtcctcaccgtcctgcaccaggactggctgaatggcaaggagtacaagtgcaaggtctccaacaaagccctcccagcccccatcgagaaaaccatctccaaagccaaaggccagccccgggaaccacaggtgtacaccctgcccccatcccgggaggagatgaccaagaaccaggtcagcctgacctgcctggtcaaaggcttctatcccagcgacatcgccgtggagtgggagagcaatggccagcccgagaacaactacaagaccacccctcccgtgctggactccgacggctccttcttcctctacagcaagctcaccgtggacaagagcaggtggcagcagggcaacgtcttctcatgctccgtgatgcatgaggctctgcacaaccactacacccagaagagcctctccctgtctcccggcaaa

SEQ ID NO: 14 - protein, 470 aa, Artificial Sequence
  amino acid sequence of heavy chain of humanized TINA1 antibody, type H2
MKHLWFFLLLVAAPRWVLSQVQLVQSGAEVKKPGASVKVSCKASGYTFTTAGMQWVRQAPGQGLEWMGWINTHSGVPKYAEDFKGRVTISLDTSTSTAYLQLSSLKSEDTAVYYCARSGFGSSYWYFDVWGQGTLVTVSSASTKGPSVFPLAPSSKSTSGGTAALGCLVKDYFPEPVTVSWNSGALTSGVHTFPAVLQSSGLYSLSSVVTVPSSSLGTQTYICNVNHKPSNTKVDKRVEPKSCDKTHTCPPCPAPELLGGPSVFLFPPKPKDTLMISRTPEVTCVVVDVSHEDPEVKFNWYVDGVEVHNAKTKPREEQYNSTYRVVSVLTVLHQDWLNGKEYKCKVSNKALPAPIEKTISKAKGQPREPQVYTLPPSREEMTKNQVSLTCLVKGFYPSDIAVEWESNGQPENNYKTTPPVLDSDGSFFLYSKLTVDKSRWQQGNVFSCSVMHEALHNHYTQKSLSLSPGK

SEQ ID NO: 15 - DNA, 1410 bp, Artificial Sequence
  nucleotide sequence of heavy chain of humanized TINA1 antibody, type H3
atgaaacacctgtggttcttcctcctgctggtggcagctcccagatgggtgctgagccagatccagctggtgcagtctggcgccgaagtgaagaaacccggcgagagcgtgaaggtgtcctgcaaggccagcggctacacctttaccaccgccggcatgcagtgggtgcagcagatgcctggcaagggcctggaatggatgggctggatcaacacccacagcggcgtgcccaaatacgccgaggacttcaagggcagagtgaccttcagcctggacaccagcacctccaccgcctacctgcagctgagcagcctgaagtccgaggacaccgccgtgtactactgcgccagaagcggcttcggcagcagctactggtacttcgacgtgtggggccagggcaccctcgtgaccgtcagctcagcctccaccaagggcccaagcgtcttccccctggcaccctcctccaagagcacctctggcggcacagccgccctgggctgcctggtcaaggactacttccccgaacccgtgaccgtgagctggaactcaggcgccctgaccagcggcgtgcacaccttccccgctgtcctgcagtcctcaggactctactccctcagcagcgtggtgaccgtgccctccagcagcttgggcacccagacctacatctgcaacgtgaatcacaagcccagcaacaccaaggtggacaagagagttgagcccaaatcttgtgacaaaactcacacatgcccaccctgcccagcacctgaactcctggggggaccctcagtcttcctcttccccccaaaacccaaggacaccctcatgatctcccggacccctgaggtcacatgcgtggtggtggacgtgagccacgaagaccctgaggtcaagttcaactggtacgtggacggcgtggaggtgcataatgccaagacaaagccccgggaggagcagtacaacagcacgtaccgggtggtcagcgtcctcaccgtcctgcaccaggactggctgaatggcaaggagtacaagtgcaaggtctccaacaaagccctcccagcccccatcgagaaaaccatctccaaagccaaaggccagccccgggaaccacaggtgtacaccctgcccccatcccgggaggagatgaccaagaaccaggtcagcctgacctgcctggtcaaaggcttctatcccagcgacatcgccgtggagtgggagagcaatggccagcccgagaacaactacaagaccacccctcccgtgctggactccgacggctccttcttcctctacagcaagctcaccgtggacaagagcaggtggcagcagggcaacgtcttctcatgctccgtgatgcatgaggctctgcacaaccactacacccagaagagcctctccctgtctcccggcaaa

SEQ ID NO: 16 - protein, 470 aa, Artificial Sequence
  amino acid sequence of heavy chain of humanized TINA1 antibody, type H3
MKHLWFFLLLVAAPRWVLSQIQLVQSGAEVKKPGESVKVSCKASGYTFTTAGMQWVQQMPGKGLEWMGWINTHSGVPKYAEDFKGRVTFSLDTSTSTAYLQLSSLKSEDTAVYYCARSGFGSSYWYFDVWGQGTLVTVSSASTKGPSVFPLAPSSKSTSGGTAALGCLVKDYFPEPVTVSWNSGALTSGVHTFPAVLQSSGLYSLSSVVTVPSSSLGTQTYICNVNHKPSNTKVDKRVEPKSCDKTHTCPPCPAPELLGGPSVFLFPPKPKDTLMISRTPEVTCVVVDVSHEDPEVKFNWYVDGVEVHNAKTKPREEQYNSTYRVVSVLTVLHQDWLNGKEYKCKVSNKALPAPIEKTISKAKGQPREPQVYTLPPSREEMTKNQVSLTCLVKGFYPSDIAVEWESNGQPENNYKTTPPVLDSDGSFFLYSKLTVDKSRWQQGNVFSCSVMHEALHNHYTQKSLSLSPGK

SEQ ID NO: 17 - DNA, 702 bp, Artificial Sequence
  nucleotide sequence of light chain of humanized TINA1 antibody, type L1
atggtgctgcagacccaggtgttcatctccctgctgctgtggatctccggcgcgtacggcgacatccagatgacccagagccctagcagcctgagcgccagcgtgggcgacagagtgaccatcacatgcaaggccagccaggacgtgtccacagccgtggcctggtatcagcagaagcctggcaaggcccccaagctgctgatctacagcgccagctaccggtacaccggcgtgcccagcagattttctggcagcggctccggcaccgacttcaccctgacaatcagcagcctgcagcccgaggacttcgccgtgtactactgccagcagcactacatcacccccctgacctttggccagggcaccaagctggaaatcaagcgtacggtggccgccccctccgtgttcatcttccccccctccgacgagcagctgaagtccggcaccgcctccgtggtgtgcctgctgaataacttctaccccagagaggccaaggtgcagtggaaggtggacaacgccctgcagtccgggaactcccaggagagcgtgaccgagcaggacagcaaggacagcacctacagcctgagcagcaccctgaccctgagcaaagccgactacgagaagcacaaggtgtacgcctgcgaggtgacccaccagggcctgagctcccccgtcaccaagagcttcaacaggggggagtgt

SEQ ID NO: 18 - protein, 234 aa, Artificial Sequence
  amino acid sequence of light chain of humanized TINA1 antibody, type L1
MVLQTQVFISLLLWISGAYGDIQMTQSPSSLSASVGDRVTITCKASQDVSTAVAWYQQKPGKAPKLLIYSASYRYTGVPSRFSGSGSGTDFTLTISSLQPEDFAVYYCQQHYITPLTFGQGTKLEIKRTVAAPSVFIFPPSDEQLKSGTASVVCLLNNFYPREAKVQWKVDNALQSGNSQESVTEQDSKDSTYSLSSTLTLSKADYEKHKVYACEVTHQGLSSPVTKSFNRGEC

SEQ ID NO: 19 - DNA, 702 bp, Artificial Sequence
  nucleotide sequence of light chain of humanized TINA1 antibody, type L2
atggtgctgcagacccaggtgttcatctccctgctgctgtggatctccggcgcgtacggcgacatcgtgatgacccagagccctagcagcctgagcgccagcgtgggcgacagagtgaccatcacatgcaaggccagccaggacgtgtccacagccgtggcctggtatcagcagaagcctggcaaggcccccaagctgctgatctacagcgccagctaccggtacaccggcgtgcccagcagattttctggcagcggctccggcaccgacttcaccctgacaatcagcagcctgcagcccgaggacttcgccgtgtactactgccagcagcactacatcacccccctgacctttggccagggcaccaagctggaaatcaagcgtacggtggccgccccctccgtgttcatcttccccccctccgacgagcagctgaagtccggcaccgcctccgtggtgtgcctgctgaataacttctaccccagagaggccaaggtgcagtggaaggtggacaacgccctgcagtccgggaactcccaggagagcgtgaccgagcaggacagcaaggacagcacctacagcctgagcagcaccctgaccctgagcaaagccgactacgagaagcacaaggtgtacgcctgcgaggtgacccaccagggcctgagctcccccgtcaccaagagcttcaacaggggggagtgt

SEQ ID NO: 20 - protein, 234 aa, Artificial Sequence
  amino acid sequence of light chain of humanized TINA1 antibody, type L2
MVLQTQVFISLLLWISGAYGDIVMTQSPSSLSASVGDRVTITCKASQDVSTAVAWYQQKPGKAPKLLIYSASYRYTGVPSRFSGSGSGTDFTLTISSLQPEDFAVYYCQQHYITPLTFGQGTKLEIKRTVAAPSVFIFPPSDEQLKSGTASVVCLLNNFYPREAKVQWKVDNALQSGNSQESVTEQDSKDSTYSLSSTLTLSKADYEKHKVYACEVTHQGLSSPVTKSFNRGEC

SEQ ID NO: 21 - DNA, 702 bp, Artificial Sequence
  nucleotide sequence of light chain of humanized TINA1 antibody, type L3
atggtgctgcagacccaggtgttcatctccctgctgctgtggatctccggcgcgtacggcgacatcgtgatgacccagagccctagcagcctgagcgccagcgtgggcgacagagtgaccatcacatgcaaggccagccaggacgtgtccacagccgtggcctggtatcagcagaagcccggcaagcagcccaagctgctgatctacagcgccagctaccggtacaccggcgtgcccagcagattttctggcagcggctccggcaccgacttcaccctgacaatcagcagcctgcagcccgaggacttcgccgtgtactactgccagcagcactacatcacccccctgacctttggccagggcaccaagctggaaatcaagcgtacggtggccgccccctccgtgttcatcttccccccctccgacgagcagctgaagtccggcaccgcctccgtggtgtgcctgctgaataacttctaccccagagaggccaaggtgcagtggaaggtggacaacgccctgcagtccgggaactcccaggagagcgtgaccgagcaggacagcaaggacagcacctacagcctgagcagcaccctgaccctgagcaaagccgactacgagaagcacaaggtgtacgcctgcgaggtgacccaccagggcctgagctcccccgtcaccaagagcttcaacaggggggagtgt

SEQ ID NO: 22 - protein, 234 aa, Artificial Sequence
  amino acid sequence of light chain of humanized TINA1 antibody, type L3
MVLQTQVFISLLLWISGAYGDIVMTQSPSSLSASVGDRVTITCKASQDVSTAVAWYQQKPGKQPKLLIYSASYRYTGVPSRFSGSGSGTDFTLTISSLQPEDFAVYYCQQHYITPLTFGQGTKLEIKRTVAAPSVFIFPPSDEQLKSGTASVVCLLNNFYPREAKVQWKVDNALQSGNSQESVTEQDSKDSTYSLSSTLTLSKADYEKHKVYACEVTHQGLSSPVTKSFNRGEC

SEQ ID NO: 23 - protein, 5 aa, Mus musculus
TAGMQ

SEQ ID NO: 24 - protein, 17 aa, Mus musculus
WINTHSGVPKYAEDFKG

SEQ ID NO: 25 - protein, 12 aa, Mus musculus
SGFGSSYWYFDV

SEQ ID NO: 26 - protein, 11 aa, Mus musculus
KASQDVSTAVA

SEQ ID NO: 27 - protein, 7 aa, Mus musculus
SASYRYT

SEQ ID NO: 28 - protein, 9 aa, Mus musculus
QQHYITPLT

SEQ ID NO: 29 - DNA, 1410 bp, Homo sapiens
atgaaacacctgtggttcttcctcctgctggtggcagctcccagatgggtgctgagccaggtgcagctgcagcagagcggcagcgagctgaagaagcctggcgccagcgtcaaggtgtcctgcaaggccagcggctacaccttcaccaactacggcatgaactgggtgaagcaggccccaggccagggcctgaagtggatgggctggatcaacacctacaccggcgagcccacctacaccgacgacttcaagggccggttcgccttcagcctggacaccagcgtgagcaccgcctacctgcagatcagcagcctgaaggccgacgataccgccgtgtacttctgcgccagaggcggcttcggcagcagctactggtacttcgacgtgtggggccagggcagcctggtgaccgtgagctcagcctccaccaagggcccaagcgtcttccccctggcaccctcctccaagagcacctctggcggcacagccgccctgggctgcctggtcaaggactacttccccgaacccgtgaccgtgagctggaactcaggcgccctgaccagcggcgtgcacaccttccccgctgtcctgcagtcctcaggactctactccctcagcagcgtggtgaccgtgccctccagcagcttgggcacccagacctacatctgcaacgtgaatcacaagcccagcaacaccaaggtggacaagagagttgagcccaaatcttgtgacaaaactcacacatgcccaccctgcccagcacctgaactcctggggggaccctcagtcttcctcttccccccaaaacccaaggacaccctcatgatctcccggacccctgaggtcacatgcgtggtggtggacgtgagccacgaagaccctgaggtcaagttcaactggtacgtggacggcgtggaggtgcataatgccaagacaaagccccgggaggagcagtacaacagcacgtaccgggtggtcagcgtcctcaccgtcctgcaccaggactggctgaatggcaaggagtacaagtgcaaggtctccaacaaagccctcccagcccccatcgagaaaaccatctccaaagccaaaggccagccccgggaaccacaggtgtacaccctgcccccatcccgggaggagatgaccaagaaccaggtcagcctgacctgcctggtcaaaggcttctatcccagcgacatcgccgtggagtgggagagcaatggccagcccgagaacaactacaagaccacccctcccgtgctggactccgacggctccttcttcctctacagcaagctcaccgtggacaagagcaggtggcagcagggcaacgtcttctcatgctccgtgatgcatgaggctctgcacaaccactacacccagaagagcctctccctgtctcccggcaaa

SEQ ID NO: 30 - protein, 470 aa, Homo sapiens
MKHLWFFLLLVAAPRWVLSQVQLQQSGSELKKPGASVKVSCKASGYTFTNYGMNWVKQAPGQGLKWMGWINTYTGEPTYTDDFKGRFAFSLDTSVSTAYLQISSLKADDTAVYFCARGGFGSSYWYFDVWGQGSLVTVSSASTKGPSVFPLAPSSKSTSGGTAALGCLVKDYFPEPVTVSWNSGALTSGVHTFPAVLQSSGLYSLSSVVTVPSSSLGTQTYICNVNHKPSNTKVDKRVEPKSCDKTHTCPPCPAPELLGGPSVFLFPPKPKDTLMISRTPEVTCVVVDVSHEDPEVKFNWYVDGVEVHNAKTKPREEQYNSTYRVVSVLTVLHQDWLNGKEYKCKVSNKALPAPIEKTISKAKGQPREPQVYTLPPSREEMTKNQVSLTCLVKGFYPSDIAVEWESNGQPENNYKTTPPVLDSDGSFFLYSKLTVDKSRWQQGNVFSCSVMHEALHNHYTQKSLSLSPGK

SEQ ID NO: 31 - DNA, 702 bp, Homo sapiens
atggtgctgcagacccaggtgttcatctccctgctgctgtggatctccggcgcgtacggcgatatccagctgacccagagccccagcagcctgagcgccagcgtgggcgacagagtgtccatcacatgcaaggccagccaggacgtgtccattgccgtggcctggtatcagcagaagcccggcaaggcccccaagctgctgatctacagcgccagctaccggtacaccggcgtgcccgacagattcagcggcagcggctccggcaccgacttcaccctgaccatcagcagcctgcagcccgaggacttcgccgtgtactactgccagcagcactacatcacccccctgaccttcggagccggcaccaaggtggaaatcaagcgtacggtggccgccccctccgtgttcatcttccccccctccgacgagcagctgaagtccggcaccgcctccgtggtgtgcctgctgaataacttctaccccagagaggccaaggtgcagtggaaggtggacaacgccctgcagtccgggaactcccaggagagcgtgaccgagcaggacagcaaggacagcacctacagcctgagcagcaccctgaccctgagcaaagccgactacgagaagcacaaggtgtacgcctgcgaggtgacccaccagggcctgagctcccccgtcaccaagagcttcaacaggggggagtgt

SEQ ID NO: 32 - protein, 234 aa, Homo sapiens
MVLQTQVFISLLLWISGAYGDIQLTQSPSSLSASVGDRVSITCKASQDVSIAVAWYQQKPGKAPKLLIYSASYRYTGVPDRFSGSGSGTDFTLTISSLQPEDFAVYYCQQHYITPLTFGAGTKVEIKRTVAAPSVFIFPPSDEQLKSGTASVVCLLNNFYPREAKVQWKVDNALQSGNSQESVTEQDSKDSTYSLSSTLTLSKADYEKHKVYACEVTHQGLSSPVTKSFNRGEC

SEQ ID NO: 33 - DNA, 30 bp, Artificial Sequence
  nucleotide sequence of primer mG2aVR2
agagttccaggtcaaggtcactggctcagg

SEQ ID NO: 34 - DNA, 30 bp, Artificial Sequence
  nucleotide sequence of primer mKVR2
agtccaactgttcaggacgccattttgtcg

SEQ ID NO: 35 - DNA, 30 bp, Artificial Sequence
  nucleotide sequence of primer 3.3-F1
tataccgtcgacctctagctagagcttggc

SEQ ID NO: 36 - DNA, 30 bp, Artificial Sequence
  nucleotide sequence of primer 3.3-R1
gctatggcagggcctgccgccccgacgttg

SEQ ID NO: 37 - DNA, 47 bp, Artificial Sequence
  nucleotide sequence of primer TINA1H-F
ccagatgggtgctgagccagatccagttggtgcagtctggacctgag

SEQ ID NO: 38 - DNA, 48 bp, Artificial Sequence
  nucleotide sequence of primer TINA1H-R
cttggtggaggctgagctgacggtgaccgcggtccctgcgccccagac

SEQ ID NO: 39 - DNA, 48 bp, Artificial Sequence
  nucleotide sequence of primer TINA1L-F
atctccggcgcgtacggcgacattgtgatgacccagtctcacaaattc

SEQ ID NO: 40 - DNA, 45 bp, Artificial Sequence
  nucleotide sequence of primer TINA1L-R
ggagggggcggccacagcccgtttcagctccagcttggtcccagc

SEQ ID NO: 41 - DNA, 22 bp, Artificial Sequence
  nucleotide sequence of primer EG-Inf-F
agctcccagatgggtgctgagc

SEQ ID NO: 42 - DNA, 22 bp, Artificial Sequence
  nucleotide sequence of primer EG1-Inf-R
gggcccttggtggaggctgagc

SEQ ID NO: 43 - DNA, 24 bp, Artificial Sequence
  nucleotide sequence of primer CM-LKF
ctgtggatctccggcgcgtacggc

SEQ ID NO: 44 - DNA, 21 bp, Artificial Sequence
  nucleotide sequence of primer KCL-Inf-R
ggagggggcggccaccgtacg

SEQ ID NO: 45 - protein, 4 aa, Artificial Sequence
  Amino acid sequence of Lp
DGGF

SEQ ID NO: 46 - protein, 4 aa, Artificial Sequence
  Amino acid sequence of Lp
EGGF

SEQ ID NO: 47 - protein, 4 aa, Artificial Sequence
  Amino acid sequence of Lp
GGFG

SEQ ID NO: 48 - protein, 4 aa, Artificial Sequence
  Amino acid sequence of Lp
SGGF

SEQ ID NO: 49 - protein, 4 aa, Artificial Sequence
  Amino acid sequence of Lp
KGGF

SEQ ID NO: 50 - protein, 5 aa, Artificial Sequence
  Amino acid sequence of Lp
DGGFG

SEQ ID NO: 51 - protein, 5 aa, Artificial Sequence
  Amino acid sequence of Lp
GGFGG

SEQ ID NO: 52 - protein, 6 aa, Artificial Sequence
  Amino acid sequence of Lp
DDGGFG

SEQ ID NO: 53 - protein, 6 aa, Artificial Sequence
  Amino acid sequence of Lp
KDGGFG

SEQ ID NO: 54 - protein, 7 aa, Artificial Sequence
  Amino acid sequence of Lp
GGFGGGF